European Patent Specification EP 4 092 123 B1, published June 11, 2025. Title: Novel transcriptional regulator variant and a method for producing L-valine using the same. Applicant: CJ CheilJedang Corporation. The sequence listing filed with the application follows.

SEQUENCE LISTING (10 sequences)

SEQ ID NO: 1 - protein, 253 aa, Artificial Sequence
  transcriptional regulator iolR variant
MTTEAPIWPAELFEDLDRNGPIPLYFQVAQRLEDGIRSGVLPPGARLENEISVAKHLNVSRPTVRRAIQEVVDKGLLVRRRGVGTQVVQSHVTRPVELTSFFNDLKNANLDPKTRVLEHRLLAASSAIAEKLGVSAGDEVLLIRRLRSTGDIPVAILENYLPPAFNDVSLDELEKGGLYDALRSRGVVLKIANQKIGARRAVGEESTLLDIEDGGPLLTVERVALDNSGQVIELGSHCYRPDMYNFKTTLVAR

SEQ ID NO: 2 - DNA, 762 bp, Artificial Sequence
  transcriptional regulator iolR variant coding gene
atgaccaccgaagctcccatttggccagccgaactcttcgaagacctcgaccgcaacggaccaatccccctctacttccaagtagcccaacgcctcgaagacggcatccgcagtggagtcctcccacccggagcacgcctagaaaacgagatctccgtggcgaaacacctcaacgtatcccgccccaccgtccgccgcgccatccaagaagtcgtagacaaaggcctcctagttcgtcgccgcggtgttggcacccaggtcgtccaaagccacgtcacccgcccagtcgaactgaccagtttcttcaacgacctcaaaaacgccaacctggaccccaaaacccgagtcctcgagcaccgcctccttgctgcaagttccgccatcgcagaaaaactcggagtttccgcaggtgacgaagtcctcctcatccgccgcctccgctccaccggagacatccccgtagcgatcctggaaaactacctccccccagcattcaacgacgtctccctcgacgaactggaaaaaggcggactctacgatgcactgcgcagccgtggcgttgtcctaaaaatcgccaaccagaaaatcggtgcgcgccgagcagtcggtgaagaaagcaccctcctcgacatcgaagacggcggaccacttctcaccgtcgaacgcgttgcattggataattccggccaagtaatcgagttgggaagccactgctaccgcccagatatgtacaactttaaaaccactctggtggccaggtaa

SEQ ID NO: 3 - protein, 253 aa, Artificial Sequence
  Wild-type transcriptional regulator iolR
MTTEAPIWPAELFEDLDRNGPIPLYFQVAQRLEDGIRSGVLPPGARLENEISVAKHLNVSRPTVRRAIQEVVDKGLLVRRRGVGTQVVQSHVTRPVELTSFFNDLKNANLDPKTRVLEHRLLAASSAIAEKLGVSAGDEVLLIRRLRSTGDIPVAILENYLPPAFNDVSLDELEKGGLYDALRSRGVVLKIANQKIGARRAVGEESTLLDIEDGGPLLTVERVALDNSGQVIELGSHCYRPDMYNFETTLVAR

SEQ ID NO: 4 - DNA, 762 bp, Artificial Sequence
  Wild-type transcriptional regulator iolR coding gene
atgaccaccgaagctcccatttggccagccgaactcttcgaagacctcgaccgcaacggaccaatccccctctacttccaagtagcccaacgcctcgaagacggcatccgcagtggagtcctcccacccggagcacgcctagaaaacgagatctccgtggcgaaacacctcaacgtatcccgccccaccgtccgccgcgccatccaagaagtcgtagacaaaggcctcctagttcgtcgccgcggtgttggcacccaggtcgtccaaagccacgtcacccgcccagtcgaactgaccagtttcttcaacgacctcaaaaacgccaacctggaccccaaaacccgagtcctcgagcaccgcctccttgctgcaagttccgccatcgcagaaaaactcggagtttccgcaggtgacgaagtcctcctcatccgccgcctccgctccaccggagacatccccgtagcgatcctggaaaactacctccccccagcattcaacgacgtctccctcgacgaactggaaaaaggcggactctacgatgcactgcgcagccgtggcgttgtcctaaaaatcgccaaccagaaaatcggtgcgcgccgagcagtcggtgaagaaagcaccctcctcgacatcgaagacggcggaccacttctcaccgtcgaacgcgttgcattggataattccggccaagtaatcgagttgggaagccactgctaccgcccagatatgtacaactttgaaaccactctggtggccaggtaa

SEQ ID NO: 5 - DNA, 40 bp, Artificial Sequence
  iolR_1F
tgaattcgagctcggtacccccaagaagtcgtagacaaag

SEQ ID NO: 6 - DNA, 33 bp, Artificial Sequence
  iolR_2R
gccaccagagtggttttaaagttgtacatatct

SEQ ID NO: 7 - DNA, 33 bp, Artificial Sequence
  iolR_3F
agatatgtacaactttaaaaccactctggtggc

SEQ ID NO: 8 - DNA, 40 bp, Artificial Sequence
  iolR_4R
gtcgactctagaggatccccttgagctaagtatcctatga

SEQ ID NO: 9 - DNA, 20 bp, Artificial Sequence
  iolR_5F
ccaagaagtcgtagacaaag

SEQ ID NO: 10 - DNA, 20 bp, Artificial Sequence
  iolR_6R
ttgagctaagtatcctatga